European Patent Application EP 4 424 702 A1, published September 4, 2024. Title: FULLY GENETICALLY ENCODED NAD+PROTEIN PROBE BASED ON RESONANCE ENERGY TRANSFER,AND PREPARATION METHOD THEREFOR AND USE THEREOF. Applicant: SHENZHEN INSTITUTES OF ADVANCED TECHNOLOGY. The sequence listing filed with the application follows.

SEQUENCE LISTING (13 sequences)

SEQ ID NO: 1 - protein, 716 aa, (Artificial Sequence)
MVSKGEAVIKEFMRFKVHMEGSMNGHEFEIEGEGEGRPYEGTQTAKLKVTKGGPLPFSWDILSPQFMYGSRAFTKHPADIPDYYKQSFPEGFKWERVMNFEDGGAVTVTQDTSLEDGTLIYKVKLRGTNFPPDGPVMQKKTMGWEASTERLYPEDGVLKGDIKMALRLKDGGRYLADFKTTYKAKKPVQMPGAYNVDRKLDITSHNEDYTVVEQYERSEGRHSTLTLTAATTRAQELRKQLNQYSHEYYVKDQPSVEDYVYDRLYKELVDIETEFPDLITPDSPTQNVGGKVLSGFEKAPHDIPMYSLNDGFSKEDIFAFDERVRKAIGKPVAYCCELLIDGLAISLRYENGVFVRGATRGDGTVGENITENLRTVRSVPMDLTEPISVEVRGECYMPKQSFVALNEEREENGQDIFANPRNAAAGSLRQLDTKIVAKRNLNTFLYTVADFGPMKAKTQFEALEELSAIGFRTNPERQLCQSIDEVWAYIEEYHEKRSTLPYEINGIVIKVNEFALQDELGFTVKAPRWAIAYKFPGDQMGQIEKIFKVVYPVDDHHFKVILHYGTLVIDGVTPNMIDYFGRPYEGIAVFDGKKITVTGTLWNGNKIIDERLINPDGSLLFRVTINGVTGWRLCERILAGGTGGSGGTGGSMVFTLEDFVGDWRQTAGYNLDQVLEQGGVSSLFQNLGVSVTPIQRIVLSGENGLKIDIHVIIPYE

SEQ ID NO: 2 - protein, 224 aa, (Artificial Sequence)
MVSKGEAVIKEFMRFKVHMEGSMNGHEFEIEGEGEGRPYEGTQTAKLKVTKGGPLPFSWDILSPQFMYGSRAFTKHPADIPDYYKQSFPEGFKWERVMNFEDGGAVTVTQDTSLEDGTLIYKVKLRGTNFPPDGPVMQKKTMGWEASTERLYPEDGVLKGDIKMALRLKDGGRYLADFKTTYKAKKPVQMPGAYNVDRKLDITSHNEDYTVVEQYERSEGRHST

SEQ ID NO: 3 - protein, 312 aa, (Artificial Sequence)
LTLTAATTRAQELRKQLNQYSHEYYVKDQPSVEDYVYDRLYKELVDIETEFPDLITPDSPTQNVGGKVLSGFEKAPHDIPMYSLNDGFSKEDIFAFDERVRKAIGKPVAYCCELLIDGLAISLRYENGVFVRGATRGDGTVGENITENLRTVRSVPMDLTEPISVEVRGECYMPKQSFVALNEEREENGQDIFANPRNAAAGSLRQLDTKIVAKRNLNTFLYTVADFGPMKAKTQFEALEELSAIGFRTNPERQLCQSIDEVWAYIEEYHEKRSTLPYEINGIVIKVNEFALQDELGFTVKAPRWAIAYKFP

SEQ ID NO: 4 - protein, 180 aa, (Artificial Sequence)
GDQMGQIEKIFKVVYPVDDHHFKVILHYGTLVIDGVTPNMIDYFGRPYEGIAVFDGKKITVTGTLWNGNKIIDERLINPDGSLLFRVTINGVTGWRLCERILAGGTGGSGGTGGSMVFTLEDFVGDWRQTAGYNLDQVLEQGGVSSLFQNLGVSVTPIQRIVLSGENGLKIDIHVIIPYE

SEQ ID NO: 5 - protein, 716 aa, (Artificial Sequence)
MVSKGEAVIKEFMRFKVHMEGSMNGHEFEIEGEGEGRPYEGTQTAKLKVTKGGPLPFSWDILSPQFMYGSRAFTKHPADIPDYYKQSFPEGFKWERVMNFEDGGAVTVTQDTSLEDGTLIYKVKLRGTNFPPDGPVMQKKTMGWEASTERLYPEDGVLKGDIKMALRLKDGGRYLADFKTTYKAKKPVQMPGAYNVDRKLDITSHNEDYTVVEQYERSEGRHSTLTLTAATTRAQELRKQLNQYSHEYYVKDQPSVEDYVYDRLYKELVDIETEFPDLITPDSPTQNVGGKVLSGFEKAPHDIPMYSLNDGFSKEDIFAFDERVRKAIGKPVAYCCELLIDGLAISLRYENGVFVRGATRGDGTVGENITENLRTVRSVPMPLTEPISVEVRGECYMPKQSFVALNEEREENGQDIFANPRNAAAGSLRQLDTKIVAKRNLNTFLYTVADFGPMKAKTQFEALEELSAIGFRTNPERQLCQSIDEVWAYIEEYHEKRSTLPYEINGIVIKVNEFALQDELGFTVKAPRWAIAYKFPGDQMGQIEKIFKVVYPVDDHHFKVILHYGTLVIDGVTPNMIDYFGRPYEGIAVFDGKKITVTGTLWNGNKIIDERLINPDGSLLFRVTINGVTGWRLCERILAGGTGGSGGTGGSMVFTLEDFVGDWRQTAGYNLDQVLEQGGVSSLFQNLGVSVTPIQRIVLSGENGLKIDIHVIIPYE

SEQ ID NO: 6 - protein, 296 aa, (Artificial Sequence)
LNQYSHEYYVKDQPSVEDYVYDRLYKELVDIETEFPDLITPDSPTQNVGGKVLSGFEKAPHDIPMYSLNDGFSKEDIFAFDERVRKAIGKPVAYCCELLIDGLAISLRYENGVFVRGATRGDGTVGENITENLRTVRSVPMPLTEPISVEVRGECYMPKQSFVALNEEREENGQDIFANPRNAAAGSLRQLDTKIVAKRNLNTFLYTVADFGPMKAKTQFEALEELSAIGFRTNPERQLCQSIDEVWAYIEEYHEKRSTLPYEINGIVIKVNEFALQDELGFTVKAPRWAIAYKFP

SEQ ID NO: 7 - protein, 716 aa, (Artificial Sequence)
MVSKGEAVIKEFMRFKVHMEGSMNGHEFEIEGEGEGRPYEGTQTAKLKVTKGGPLPFSWDILSPQFMYGSRAFTKHPADIPDYYKQSFPEGFKWERVMNFEDGGAVTVTQDTSLEDGTLIYKVKLRGTNFPPDGPVMQKKTMGWEASTERLYPEDGVLKGDIKMALRLKDGGRYLADFKTTYKAKKPVQMPGAYNVDRKLDITSHNEDYTVVEQYERSEGRHSTLTLTAATTRAQELRKQLNQYSHEYYVKDQPSVEDYVYDRLYKELVDIETEFPDLITPDSPTQNVGGKVLSGFEKAPHDIPMYSLNDGFSKEDIFAFDERVRKAIGKPVAYCCELLIDGLAISLRYENGVFVRGATRGDGTVGENITENLRTVRSVPMDLTEPISVEVRGECYMPKQSFVALNEEREENGQDIFANPRNAAAGSLRQLDTKIVAKRNLNTFLYTVADFGPMKAKTQFEALEELSAIGFRTNPERQLCQSIDEVWAYIEEYHEKRSTLPYEINGIVIKVNEFALQDELGFTVKAPRWAIAYKFPVDQMGQIEKIFKVVYPVDDHHFKVILHYGTLVIDGVTPNMIDYFGRPYEGIAVFDGKKITVTGTLWNGNKIIDERLINPDGSLLFRVTINGVTGWRLCERILAGGTGGSGGTGGSMVFTLEDFVGDWRQTAGYNLDQVLEQGGVSSLFQNLGVSVTPIQRIVLSGENGLKIDIHVIIPYE

SEQ ID NO: 8 - protein, 180 aa, (Artificial Sequence)
VDQMGQIEKIFKVVYPVDDHHFKVILHYGTLVIDGVTPNMIDYFGRPYEGIAVFDGKKITVTGTLWNGNKIIDERLINPDGSLLFRVTINGVTGWRLCERILAGGTGGSGGTGGSMVFTLEDFVGDWRQTAGYNLDQVLEQGGVSSLFQNLGVSVTPIQRIVLSGENGLKIDIHVIIPYE

SEQ ID NO: 9 - protein, 711 aa, (Artificial Sequence)
MASLPATHELHIFGSINGVDFDMVGQGTGNPNDGYEELNLKSTKGDLQFSPWILVPHIGYGFHQYLPYPDGMSPFQAAMVDGSGYQVHRTMQFEDGASLTVNYRYTYEGSHIKGEAQVKGTGFPADGPVMTNSLTAADWCRSKKTYPNDKTIISTFKWSYTTGNGKRYRSTARTTYTFAKPMAANYLKNQPMYVFRKTELKHSKTELNFKEWQKAFTDKLTLTAATTRAQELRKQLNQYSHEYYVKDQPSVEDYVYDRLYKELVDIETEFPDLITPDSPTQNVGGKVLSGFEKAPHDIPMYSLNDGFSKEDIFAFDERVRKAIGKPVAYCCELLIDGLAISLRYENGVFVRGATRGDGTVGENITENLRTVRSVPMDLTEPISVEVRGECYMPKQSFVALNEEREENGQDIFANPRNAAAGSLRQLDTKIVAKRNLNTFLYTVADFGPMKAKTQFEALEELSAIGFRTNPERQLCQSIDEVWAYIEEYHEKRSTLPYEINGIVIKVNEFALQDELGFTVKAPRWAIAYKFPVDQMGQIEKIFKVVYPVDDHHFKVILHYGTLVIDGVTPNMIDYFGRPYEGIAVFDGKKITVTGTLWNGNKIIDERLINPDGSLLFRVTINGVTGWRLCERILAGGTGGSGGTGGSMVFTLEDFVGDWRQTAGYNLDQVLEQGGVSSLFQNLGVSVTPIQRIVLSGENGLKIDIHVIIPYE

SEQ ID NO: 10 - protein, 219 aa, (Artificial Sequence)
MASLPATHELHIFGSINGVDFDMVGQGTGNPNDGYEELNLKSTKGDLQFSPWILVPHIGYGFHQYLPYPDGMSPFQAAMVDGSGYQVHRTMQFEDGASLTVNYRYTYEGSHIKGEAQVKGTGFPADGPVMTNSLTAADWCRSKKTYPNDKTIISTFKWSYTTGNGKRYRSTARTTYTFAKPMAANYLKNQPMYVFRKTELKHSKTELNFKEWQKAFTDK

SEQ ID NO: 11 - protein, 760 aa, (Artificial Sequence)
MVSKGEAVIKEFMRFKVHMEGSMNGHEFEIEGEGEGRPYEGTQTAKLKVTKGGPLPFSWDILSPQFMYGSRAFTKHPADIPDYYKQSFPEGFKWERVMNFEDGGAVTVTQDTSLEDGTLIYKVKLRGTNFPPDGPVMQKKTMGWEASTERLYPEDGVLKGDIKMALRLKDGGRYLADFKTTYKAKKPVQMPGAYNVDRKLDITSHNEDYTVVEQYERSEGRHLTLTLTAATTRAQELRKQLNQYSHEYYVKDQPSVEDYVYDRLYKELVDIETEFPDLITPDSPTQNVGGKVLSGFEKAPHDIPMYSLNDGFSKEDIFAFDERVRKAIGKPVAYCCELLIDGLAISLRYENGVFVRGATRGDGTVGENITENLRTVRSVPMDLTEPISVEVRGECYMPKQSFVALNEEREENGQDIFANPRNAAAGSLRQLDTKIVAKRNLNTFLYTVADFGPMKAKTQFEALEELSAIGFRTNPERQLCQSIDEVWAYIEEYHEKRSTLPYEINGIVIKVNEFALQDELGFTVKAPRWAIAYKFPPPATHELHIFGSINGVDFDMVGQGTGNPNDGYEELNLKSTKGDLQFSPWILVPHIGYGFHQYLPYPDGMSPFQAAMVDGSGYQVHRTMQFEDGASLTVNYRYTYEGSHIKGEAQVKGTGFPADGPVMTNSLTAADWCRSKKTYPNDKTIISTFKWSYTTGNGKRYRSTARTTYTFAKPMAANYLKNQPMYVFRKTELKHSKTELNFKEWQKAFTDVMGMDELYK

SEQ ID NO: 12 - protein, 224 aa, (Artificial Sequence)
MVSKGEAVIKEFMRFKVHMEGSMNGHEFEIEGEGEGRPYEGTQTAKLKVTKGGPLPFSWDILSPQFMYGSRAFTKHPADIPDYYKQSFPEGFKWERVMNFEDGGAVTVTQDTSLEDGTLIYKVKLRGTNFPPDGPVMQKKTMGWEASTERLYPEDGVLKGDIKMALRLKDGGRYLADFKTTYKAKKPVQMPGAYNVDRKLDITSHNEDYTVVEQYERSEGRHLT

SEQ ID NO: 13 - protein, 224 aa, (Artificial Sequence)
PPATHELHIFGSINGVDFDMVGQGTGNPNDGYEELNLKSTKGDLQFSPWILVPHIGYGFHQYLPYPDGMSPFQAAMVDGSGYQVHRTMQFEDGASLTVNYRYTYEGSHIKGEAQVKGTGFPADGPVMTNSLTAADWCRSKKTYPNDKTIISTFKWSYTTGNGKRYRSTARTTYTFAKPMAANYLKNQPMYVFRKTELKHSKTELNFKEWQKAFTDVMGMDELYK